European Patent Application EP 4 413 867 A1, published August 14, 2024. Title: Composition for raising fish. Applicant: 住友化学株式会社. The sequence listing filed with the application follows.

SEQUENCE LISTING (63 sequences)

SEQ ID NO: 1 - protein, 23 aa, Lactobacillus plantarum
KSSAYSLQMGATAIKQVKKLFKK

SEQ ID NO: 2 - protein, 22 aa, Lactobacillus plantarum
FGKSVRHVVDAIGSVAGIRGIL

SEQ ID NO: 3 - protein, 23 aa, Lactobacillus plantarum
VFHAYSARGVRNNYKSAVGPADW

SEQ ID NO: 4 - protein, 22 aa, Lactobacillus plantarum
GAWKNFWSSLRKGFYDGEAGRA

SEQ ID NO: 5 - protein, 32 aa, Lactobacillus plantarum
RRSRKNGIGYAIGYAFGAVERAVLGGSRDYNK

SEQ ID NO: 6 - protein, 28 aa, Lactobacillus plantarum
DLTTKLWSSWGYYLGKKARWNLKHPYVQ

SEQ ID NO: 7 - protein, 34 aa, Lactobacillus plantarum
SVPTSVYTLGIKILWSAYKHRKTIEKSFNKGFYH

SEQ ID NO: 8 - DNA, 171 bp, Lactobacillus plantarum
  mat_peptide 70..168
  source 1..171: mol_type = genomic DNA; note = NITE BP-03198
atgctacagtttgagaagttacaatattccaggttgccgcaaaaaaagcttgccaaaatatctggtggttttaatcggggcggttataactttggtaaaagtgttcgacatgttgttgatgcaattggttcagttgcaggcattcgtggtattttgaaaagtattcgttaa

SEQ ID NO: 9 - protein, 56 aa, Lactobacillus plantarum
  source 1..56: note = NITE BP-03198
MLQFEKLQYSRLPQKKLAKISGGFNRGGYNFGKSVRHVVDAIGSVAGIRGILKSIR

SEQ ID NO: 10 - DNA, 159 bp, Lactobacillus plantarum
  mat_peptide 55..156
  source 1..159: mol_type = genomic DNA; note = NITE BP-03198
atgaaaaaatttctagttttgcgtgaccgtgaattaaatgctatttcaggtggcgttttccatgcctatagcgcgcgtggcgttcggaataattataaaagtgctgttgggcctgccgattgggtcattagcgctgtccgaggattcatccacggatag

SEQ ID NO: 11 - protein, 52 aa, Lactobacillus plantarum
  source 1..52: note = NITE BP-03198
MKKFLVLRDRELNAISGGVFHAYSARGVRNNYKSAVGPADWVISAVRGFIHG

SEQ ID NO: 12 - DNA, 168 bp, Lactobacillus plantarum
  mat_peptide 91..165
  source 1..168: mol_type = genomic DNA; note = NITE BP-03198
atgactgtgaacaaaatgattaaggatttggatgtagtagatgcatttgcacctatttctaataataagttgaacggggttgttgggggaggcgcttggaaaaatttctggtctagtttaagaaaaggattttatgatggcgaagctggcagagcaatccgtcgttaa

SEQ ID NO: 13 - protein, 55 aa, Lactobacillus plantarum
  source 1..55: note = NITE BP-03198
MTVNKMIKDLDVVDAFAPISNNKLNGVVGGGAWKNFWSSLRKGFYDGEAGRAIRR

SEQ ID NO: 14 - DNA, 174 bp, Lactobacillus plantarum
  mat_peptide 76..171
  source 1..174: mol_type = genomic DNA; note = NITE BP-03198
atgaaaattaaattaactgttttaaatgaatttgaagaattaactgctgacgctgaaaagaatatttctggtggccgtcggagtcgtaaaaatggaattggatacgctattggttatgcgtttggcgcggttgaacgggccgtgcttggtggttcaagggattataataagtga

SEQ ID NO: 15 - protein, 57 aa, Lactobacillus plantarum
  source 1..57: note = NITE BP-03198
MKIKLTVLNEFEELTADAEKNISGGRRSRKNGIGYAIGYAFGAVERAVLGGSRDYNK

SEQ ID NO: 16 - DNA, 144 bp, Lactobacillus plantarum
  mat_peptide 55..141
  source 1..144: mol_type = genomic DNA; note = NITE BP-03198
atggataaatttgaaaaaattagtacatctaacctagaaaagatctctggcggtgatttaacaaccaagttatggagctcttggggatattatcttggcaagaaagcacgttggaatttaaagcacccatatgttcaattttag

SEQ ID NO: 17 - protein, 47 aa, Lactobacillus plantarum
  source 1..47: note = NITE BP-03198
MDKFEKISTSNLEKISGGDLTTKLWSSWGYYLGKKARWNLKHPYVQF

SEQ ID NO: 18 - DNA, 168 bp, Lactobacillus plantarum
  mat_peptide 64..165
  source 1..168: mol_type = genomic DNA; note = NITE BP-03198
atgaataacttgaataaattttctactctaggcaagagtagcttgtctcaaattgagggcggatcagtcccaacttcagtatatacgcttggaattaaaattctatggtctgcgtataagcatcgcaaaacgattgaaaaaagttttaataaaggcttttatcattaa

SEQ ID NO: 19 - protein, 55 aa, Lactobacillus plantarum
  source 1..55: note = NITE BP-03198
MNNLNKFSTLGKSSLSQIEGGSVPTSVYTLGIKILWSAYKHRKTIEKSFNKGFYH

SEQ ID NO: 20 - DNA, 147 bp, Lactobacillus plantarum
  mat_peptide 67..144
  source 1..147: mol_type = genomic DNA; note = NITE BP-03199
atgaaaattcaaattaaaggtatgaagcaacttagtaataaggaaatgcaaaaaatagtaggtggaaagagtagtgcgtattctttgcagatgggggcaactgcaattaaacaggtaaagaaactgtttaaaaaatggggatggtaa

SEQ ID NO: 21 - protein, 48 aa, Lactobacillus plantarum
  source 1..48: note = NITE BP-03199
MKIQIKGMKQLSNKEMQKIVGGKSSAYSLQMGATAIKQVKKLFKKWGW

SEQ ID NO: 22 - DNA, 171 bp, Lactobacillus plantarum; identical to SEQ ID NO: 8
  mat_peptide 70..168
  source 1..171: mol_type = genomic DNA; note = NITE BP-03199

SEQ ID NO: 23 - protein, 56 aa, Lactobacillus plantarum; identical to SEQ ID NO: 9
  source 1..56: note = NITE BP-03199

SEQ ID NO: 24 - DNA, 159 bp, Lactobacillus plantarum; identical to SEQ ID NO: 10
  mat_peptide 55..156
  source 1..159: mol_type = genomic DNA; note = NITE BP-03199

SEQ ID NO: 25 - protein, 52 aa, Lactobacillus plantarum; identical to SEQ ID NO: 11
  source 1..52: note = NITE BP-03199

SEQ ID NO: 26 - DNA, 168 bp, Lactobacillus plantarum; identical to SEQ ID NO: 12
  mat_peptide 91..165
  source 1..168: mol_type = genomic DNA; note = NITE BP-03199

SEQ ID NO: 27 - protein, 55 aa, Lactobacillus plantarum; identical to SEQ ID NO: 13
  source 1..55: note = NITE BP-03199

SEQ ID NO: 28 - DNA, 174 bp, Lactobacillus plantarum; identical to SEQ ID NO: 14
  mat_peptide 76..171
  source 1..174: mol_type = genomic DNA; note = NITE BP-03199

SEQ ID NO: 29 - protein, 57 aa, Lactobacillus plantarum; identical to SEQ ID NO: 15
  source 1..57: note = NITE BP-03199

SEQ ID NO: 30 - DNA, 147 bp, Lactobacillus plantarum
  mat_peptide 67..144
  source 1..147: mol_type = genomic DNA; note = NITE BP-03200
atgaaaattcaaattaaaagtatgaagcaacttagtaataaggaaatgcaaaaaatagtaggtggaaagagtagtgcgtattctttgcagatgggggcaactgcaattaaacaggtaaagaaactgtttaaaaaatggggatggtaa

SEQ ID NO: 31 - protein, 48 aa, Lactobacillus plantarum
  source 1..48: note = NITE BP-03200
MKIQIKSMKQLSNKEMQKIVGGKSSAYSLQMGATAIKQVKKLFKKWGW

SEQ ID NO: 32 - DNA, 171 bp, Lactobacillus plantarum; identical to SEQ ID NO: 8
  mat_peptide 70..168
  source 1..171: mol_type = genomic DNA; note = NITE BP-03200

SEQ ID NO: 33 - protein, 56 aa, Lactobacillus plantarum; identical to SEQ ID NO: 9
  source 1..56: note = NITE BP-03200

SEQ ID NO: 34 - DNA, 159 bp, Lactobacillus plantarum; identical to SEQ ID NO: 10
  mat_peptide 55..156
  source 1..159: mol_type = genomic DNA; note = NITE BP-03200

SEQ ID NO: 35 - protein, 52 aa, Lactobacillus plantarum; identical to SEQ ID NO: 11
  source 1..52: note = NITE BP-03200

SEQ ID NO: 36 - DNA, 144 bp, Lactobacillus plantarum; identical to SEQ ID NO: 16
  mat_peptide 55..141
  source 1..144: mol_type = genomic DNA; note = NITE BP-03200

SEQ ID NO: 37 - protein, 47 aa, Lactobacillus plantarum; identical to SEQ ID NO: 17
  source 1..47: note = NITE BP-03200

SEQ ID NO: 38 - DNA, 168 bp, Lactobacillus plantarum; identical to SEQ ID NO: 18
  mat_peptide 64..165
  source 1..168: mol_type = genomic DNA; note = NITE BP-03200

SEQ ID NO: 39 - protein, 55 aa, Lactobacillus plantarum; identical to SEQ ID NO: 19
  source 1..55: note = NITE BP-03200

SEQ ID NO: 40 - DNA, 147 bp, Lactobacillus plantarum; identical to SEQ ID NO: 20
  mat_peptide 67..144
  source 1..147: mol_type = genomic DNA; note = NITE BP-03201

SEQ ID NO: 41 - protein, 48 aa, Lactobacillus plantarum; identical to SEQ ID NO: 21
  source 1..48: note = NITE BP-03201

SEQ ID NO: 42 - DNA, 171 bp, Lactobacillus plantarum
  mat_peptide 70..168
  source 1..171: mol_type = genomic DNA; note = NITE BP-03201
atgctacagtttgagaagttacaatattccaggttgccgcaaaaaaagcttgccaaaatatctggtggttttaatcggggcggttataactttggcaaaagtgttcgacatgttgttgatgcaattggttcagttgcaggcattcgtggtattttgaaaagtattcgttaa

SEQ ID NO: 43 - protein, 56 aa, Lactobacillus plantarum; identical to SEQ ID NO: 9
  source 1..56: note = NITE BP-03201

SEQ ID NO: 44 - DNA, 159 bp, Lactobacillus plantarum; identical to SEQ ID NO: 10
  mat_peptide 55..156
  source 1..159: mol_type = genomic DNA; note = NITE BP-03201

SEQ ID NO: 45 - protein, 52 aa, Lactobacillus plantarum; identical to SEQ ID NO: 11
  source 1..52: note = NITE BP-03201

SEQ ID NO: 46 - DNA, 168 bp, Lactobacillus plantarum; identical to SEQ ID NO: 12
  mat_peptide 91..165
  source 1..168: mol_type = genomic DNA; note = NITE BP-03201

SEQ ID NO: 47 - protein, 55 aa, Lactobacillus plantarum; identical to SEQ ID NO: 13
  source 1..55: note = NITE BP-03201

SEQ ID NO: 48 - DNA, 174 bp, Lactobacillus plantarum; identical to SEQ ID NO: 14
  mat_peptide 76..171
  source 1..174: mol_type = genomic DNA; note = NITE BP-03201

SEQ ID NO: 49 - protein, 57 aa, Lactobacillus plantarum; identical to SEQ ID NO: 15
  source 1..57: note = NITE BP-03201

SEQ ID NO: 50 - DNA, 171 bp, Lactobacillus plantarum; identical to SEQ ID NO: 8
  mat_peptide 70..168
  source 1..171: mol_type = genomic DNA; note = NITE BP-03202

SEQ ID NO: 51 - protein, 56 aa, Lactobacillus plantarum; identical to SEQ ID NO: 9
  source 1..56: note = NITE BP-03202

SEQ ID NO: 52 - DNA, 159 bp, Lactobacillus plantarum; identical to SEQ ID NO: 10
  mat_peptide 55..156
  source 1..159: mol_type = genomic DNA; note = NITE BP-03202

SEQ ID NO: 53 - protein, 52 aa, Lactobacillus plantarum; identical to SEQ ID NO: 11
  source 1..52: note = NITE BP-03202

SEQ ID NO: 54 - DNA, 168 bp, Lactobacillus plantarum; identical to SEQ ID NO: 12
  mat_peptide 91..165
  source 1..168: mol_type = genomic DNA; note = NITE BP-03202

SEQ ID NO: 55 - protein, 55 aa, Lactobacillus plantarum; identical to SEQ ID NO: 13
  source 1..55: note = NITE BP-03202

SEQ ID NO: 56 - DNA, 174 bp, Lactobacillus plantarum; identical to SEQ ID NO: 14
  mat_peptide 76..171
  source 1..174: mol_type = genomic DNA; note = NITE BP-03202

SEQ ID NO: 57 - protein, 57 aa, Lactobacillus plantarum; identical to SEQ ID NO: 15
  source 1..57: note = NITE BP-03202

SEQ ID NO: 58 - DNA, 144 bp, Lactobacillus plantarum; identical to SEQ ID NO: 16
  mat_peptide 55..141
  source 1..144: mol_type = genomic DNA; note = NITE BP-03202

SEQ ID NO: 59 - protein, 47 aa, Lactobacillus plantarum; identical to SEQ ID NO: 17
  source 1..47: note = NITE BP-03202

SEQ ID NO: 60 - DNA, 168 bp, Lactobacillus plantarum; identical to SEQ ID NO: 18
  mat_peptide 64..165
  source 1..168: mol_type = genomic DNA; note = NITE BP-03202

SEQ ID NO: 61 - protein, 55 aa, Lactobacillus plantarum; identical to SEQ ID NO: 19
  source 1..55: note = NITE BP-03202

SEQ ID NO: 62 - DNA, 174 bp, Lactococcus lactis
  mat_peptide 70..171
  source 1..174: mol_type = genomic DNA; note = NITE BP-03481
atgagtacaaaagattttaacttggatttggtatctgtttcgaagaaagattcaggtgcatcaccacgcattacaagtatttcgctatgtacacccggttgtaaaacaggagctctgatgggttgtaacatgaaaacagcaacttgtaattgtagtattcacgtaagcaaataa

SEQ ID NO: 63 - protein, 57 aa, Lactococcus lactis
  source 1..57: note = NITE BP-03481
MSTKDFNLDLVSVSKKDSGASPRITSISLCTPGCKTGALMGCNMKTATCNCSIHVSK